European Patent Specification EP 3 810 767 B1, published July 15, 2026. Title: Subtilisin Variants. Applicant: Danisco US, Inc. Alekseyev, Viktor Babe, Lilia Engin, Billur Estell, Dave Goedegebuur, Frits Kaper, Thijs Mulder, Harm Pricelius, Sina van Stigt-Thans, Sander. The sequence listing filed with the application follows.

SEQUENCE LISTING (10 sequences)

SEQ ID NO: 1 - protein, 269 aa, Bacillus gibsonii
QQTVPWGITRVQAPAVHNRGITGSGVRVAILDSGISAHEDLNIRGGASFVPGEPTTADLNGHGTHVAGTVAALNNSIGVIGVAPNAELYAVKVLGANGSGSVSGIAQGLEWAATNNMHIANMSLGSDFPSSTLERAVNYATSRDVLVIAATGNNGSGSVGYPARYANAMAVGATDQNNRRANFSQYGTGIDIVAPGVNVQSTYPGNRYVSMNGTSMATPHVAGAAALVKQRYPSWNATQIRNHLKNTATNLGNSSQFGSGLVNAEAATR

SEQ ID NO: 2 - DNA, 1052 bp, Bacillus subtilis
gcaaaacgcggatcattggaagagacgaccgtacccgcagcatcaatgcctaaaataagcggatactctctgacgatattgcctcctgcttttccggccagaccatctttgtaattaatgccggaataagcaactttaatcaggacaccatccttcggcaaatcctctgttgatatggttttcacatggactgaaacatcatcggcatttttttctgcctgcaaggcttgaaataacgttgacattcggcacactccttttcatttatatcgtaaccgaagaacgttcaaaaaaccaaatcatcaagccgccattttcacttcgccggcacattgagacaataatggacaaatccggtatcctcttcatagccgttttgctcatacaagcttcttgccttccggttgtggtgctcagtctgaagtgttaaacattttgccccgttttgccctgcataatcctttgcggcagaaagcagccggccgccggctccctttgtacgcgcatgaggaacgacaaataagtcatttaatatgtatatccttttcattgacacagaagaaaacgttggatagagctgggtaaagcctatgaattctccattttcttctgctatcaaaataacagactcgtgattttccaaacgagctttcaaaaaagcctctgccccttgcaaatcggatgcctgtctataaaattcccgatattggttaaacagcggcgcaatggcggccgcatctgatgtctttgcttggcgaatgttcatcttatttcttcctccctctcaataattttttcattctatcccttttctgtaaagtttatttttcagaatacttttatcatcatgctttgaaaaaatatcacgataatatccattgttctcacggaagcacacgcgtcgctgataaacagctgacatcaactaaaagcttcattaaatactttgaaaaaagttgttgacttaaaagaagctaaatgttatagtaataaaacagaatagtcttttaagtaagtctactctgaatttttttaaaaggagagggtaaaga

SEQ ID NO: 3 - DNA, 87 bp, Bacillus subtilis
gtgagaagcaaaaaattgtggatcagcttgttgtttgcgttaacgttaatctttacgatggcgttcagcaacatgtctgcgcaggct

SEQ ID NO: 4 - DNA, 252 bp, Bacillus lentus
gctgaagaagcaaaagaaaaatatttaattggctttaatgagcaggaagctgtcagtgagtttgtagaacaagtagaggcaaatgacgaggtcgccattctctctgaggaagaggaagtcgaaattgaattgcttcatgaatttgaaacgattcctgttttatccgttgagttaagcccagaagatgtggacgcgcttgaactcgatccagcgatttcttatattgaagaggatgcagaagtaacgacaatg

SEQ ID NO: 5 - DNA, 810 bp, Bacillus gibsonii
caacaaacagtgccatggggaattactcgtgtgcaagccccagctgttcataaccgtggaattacaggttctggtgtaagagttgctatcctcgattcaggtatttccgcacatgaagacttaaatattcgtggtggcgcaagctttgtaccaggggaaccaacgactgctgatttaaatgggcatggcacgcatgtggctgggacggtagctgctttaaacaattcgattggcgttattggcgtagcaccgaatgcggaactatacgctgttaaagtattaggggcgaatggtagcggttcggtcagcgggattgcccaaggattggaatgggcagcaacaaataacatgcacattgctaatatgagtttaggaagcgattttccaagttctacacttgagcgtgctgttaattatgcgacttctagagatgttcttgttattgcggcaactgggaataacggttctggctcagtaggctatccggcccgttatgcgaacgcaatggcagtcggagctactgaccaaaacaacagacgcgccaacttttcacagtatggcacggggattgacattgtcgcaccaggtgtaaacgtgcagagcacatacccaggtaaccgttatgtgagcatgaacggtacatcgatggctactcctcatgttgcaggtgcagcagcccttgttaaacaacgctatccatcttggaatgcgactcaaatccgcaatcatctaaagaatacggcaacgaatttaggaaactcttcacaatttggaagcggacttgtcaatgcagaagcggcaacacgctaa

SEQ ID NO: 6 - DNA, 253 bp, Bacillus amyloliquefaciens
tctagatacataaaaaaccggccttggccccgccggttttttattatttttcttcctccgcatgttcaatccgctccataatcgacggatggctccctctgaaaattttaacgagaaacggcgggttgacccggctcagtcccgtaacggccaagtcctgaaacgtctcaatcgccgcttcccggtttccggtcagctcaatgccgtaacggtcggcggcgttttcctgataccgggagacggcattcgtaat

SEQ ID NO: 7 - DNA, 855 bp, Staphylococcus aureus
ttagtgacattagaaaaccgactgtaaaaagtacagtcggcattatctcatattataaaagccagtcattaggcctatctgacaattcctgaatagagttcataaacaatcctgcatgataaccatcacaaacagaatgatgtacctgtaaagatagcggtaaatatattgaattacctttattaatgaattttcctgctgtaataatgggtagaaggtaattactattattattgatatttaagttaaacccagtaaatgaagtccatggaataatagaaagagaaaaagcattttcaggtataggtgttttgggaaacaatttccccgaaccattatatttctctacatcagaaaggtataaatcataaaactctttgaagtcattctttacaggagtccaaataccagagaatgttttagatacaccatcaaaaattgtataaagtggctctaacttatcccaataacctaactctccgtcgctattgtaaccagttctaaaagctgtatttgagtttatcacccttgtcactaagaaaataaatgcagggtaaaatttatatccttcttgttttatgtttcggtataaaacactaatatcaatttctgtggttatactaaaagtcgtttgttggttcaaataatgattaaatatctcttttctcttccaattgtctaaatcaattttattaaagttcatttgatatgcctcctaaatttttatctaaagtgaatttaggaggcttacttgtctgctttcttcattagaatcaatccttttttaaaagtcaatattactgtaacataaatatatattttaaaaatatcccactttatccaattttcgtttgt

SEQ ID NO: 8 - DNA, 994 bp, artificial sequence
  synthesized sequence - 3 prime AprE flanking sequence
tcagccttattctcctgataacgcgagacagcattagaaaaaggcgtaaccgcaaagctcaaaacagaaaacaaaagcaataacagcggaagtgccgcaagatcatgccgcccttctaaatgaaacatgctgcgggttaggcgaaccgtccgcttgtaaagcttatcaatgacataaaatccggcgagcgacacgagcaaatagccagccagaccgatgtaaacgtgcttcatgacataatggcccatttcgtggcccataataaacagaatttctgaatcgtcaagtttgttcagcgtcgtatcccacaatacaatccgtttattggccccaattcctgtaacataggcattcagcgcatttgttttttctgacatgttcacttcatatacatggtcagccggaatattggcttcatctgccagctctaaaattttgctttcaagctctttgtttttcagcggataaaaatcattgtataaaggatcgataatgaccggctgaataaaaaacagaaacagcgaaaacggcactgttaacagccaggcgtataaccaccattttttttcatgccttttgatcagccaataaaaaacgagaacgcaaagcgtaaagattggaaagctgatccaaaagctgataacctgatccttagcccagctggccgttgtctgtgtggaaatgttatagtcaagcgatacttgatagcctatccaatctaaaggcagcgtcaccaatgttgtaatcagcgaaagcacaaacacaaaaccaacggtctgcaaaaaccgaaaaggcacggccgcttcgatccatttcttgattttctttgaaacaccgctgacaagcagaacaaaaaacagaaaccaatcaagtggtaccccgataaaaaataaaaaattcttgacattcgaatactgctcggccactgccaactcagacggcttcatgaaagaagccggatcagcctgcgtccctttcacggcttccggtattg

SEQ ID NO: 9 - protein, 29 aa, Bacillus subtilis
VRSKKLWISLLFALTLIFTMAFSNMSAQA

SEQ ID NO: 10 - protein, 84 aa, Bacillus lentus
AEEAKEKYLIGFNEQEAVSEFVEQVEANDEVAILSEEEEVEIELLHEFETIPVLSVELSPEDVDALELDPAISYIEEDAEVTTM